European Patent Application EP 4 461 365 A2, published November 13, 2024. Title: Respiratory syncytial virus (RSV) vaccine. Applicant: CureVac SE. Application EP. The sequence listing filed with the application follows.

SEQUENCE LISTING (37 sequences)

SEQ ID NO: 1 - protein, 574 aa, respiratory syncytial virus
MELPILKANAITTILAAVTFCFASSQNITEEFYQSTCSAVSKGYLSALRTGWYTSVITIELSNIKENKCNGTDAKVKLINQELDKYKNAVTELQLLMQSTTAANNRARRELPRFMNYTLNNTKKTNVTLSKKRKRRFLGFLLGVGSAIASGIAVSKVLHLEGEVNKIKSALLSTNKAVVSLSNGVSVLTSKVLDLKNYIDKQLLPIVNKQSCRISNIETVIEFQQKNNRLLEITREFSVNAGVTTPVSTYMLTNSELLSLINDMPITNDQKKLMSNNVQIVRQQSYSIMSIIKEEVLAYVVQLPLYGVIDTPCWKLHTSPLCTTNTKEGSNICLTRTDRGWYCDNAGSVSFFPQAETCKVQSNRVFCDTMNSLTLPSEVNLCNVDIFNPKYDCKIMTSKTDVSSSVITSLGAIVSCYGKTKCTASNKNRGIIKTFSNGCDYVSNKGVDTVSVGNTLYYVNKQEGKSLYVKGEPIINFYDPLVFPSDEFDASISQVNEKINQSLAFIRKSDELLHHVNAGKSTTNIMITTIIIVIIVILLSLIAVGLLLYCKARSTPVTLSKDQLSGINNIAFSN

SEQ ID NO: 2 - protein, 298 aa, respiratory syncytial virus
MSKNKDQRTAKTLEKTWDTLNHLLFISSGLYKLNLKSIAQITLSILAMIISTSLIITAIIFIASANHKVTLTTAIIQDATSQIKNTTPTYLTQDPQLGISFSNLSEITSQTTTILASTTPGVKSNLQPTTVKTKNTTTTQTQPSKPTTKQRQNKPPNKPNNDFHFEVFNFVPCSICSNNPTCWAICKRIPNKKPGKKTTTKPTKKPTFKTTKKDLKPQTTKPKEVPTTKPTEEPTINTTKTNITTTLLTNNTTGNPKLTSQMETFHSTSSEGNLSPSQVSTTSEHPSQPSSPPNTTRQ

SEQ ID NO: 3 - protein, 64 aa, respiratory syncytial virus
MENTSITIEFSSKFWPYFTLIHMITTIISLLIIISIMTAILNKLCEYNVFHNKTFELPRARVNT

SEQ ID NO: 4 - protein, 256 aa, respiratory syncytial virus
METYVNKLHEGSTYTAAVQYNVLEKDDDPASLTIWVPMFQSSMPADLLIKELANVNILVKQISTPKGPSLRVMINSRSALLAQMPSKFTICANVSLDERSKLAYDVTTPCEIKACSLTCLKSKNMLTTVKDLTMKTLNPTHDIIALCEFENIVTSKKVIIPTYLRSISVRNKDLNTLENITTTEFKNAITNAKIIPYSGLLLVITVTDNKGAFKYIKPQSQFIVDLGAYLEKESIYYVTTNWKHTATRFAIKPMED

SEQ ID NO: 5 - protein, 391 aa, respiratory syncytial virus
MALSKVKLNDTLNKDQLLSSSKYTIQRSTGDSIDTPNYDVQKHINKLCGMLLITEDANHKFTGLIGMLYAMSRLGREDTIKILRDAGYHVKANGVDVTTHRQDINGKEMKFEVLTLASLTTEIQINIEIESRKSYKKMLKEMGEVAPEYRHDSPDCGMIILCIAALVITKLAAGDRSGLTAVIRRANNVLKNEMKRYKGLLPKDIANSFYEVFEKHPHFIDVFVHFGIAQSSTRGGSRVEGIFAGLFMNAYGAGQVMLRWGVLAKSVKNIMLGHASVQAEMEQVVEVYEYAQKLGGEAGFYHILNNPKASLLSLTQFPHFSSVVLGNAAGLGIMGEYRGTPRNQDLYDAAKAYAEQLKENGVINYSVLDLTAEELEAIKHQLNPKDNDVEL

SEQ ID NO: 6 - protein, 2165 aa, respiratory syncytial virus
MDPIINGNSANVYLTDSYLKGVISFSECNALGSYIFNGPYLKNDYTNLISRQNPLIEHMNLKKLNITQSLISKYHKGEIKLEEPTYFQSLLMTYKSMTSLEQIATTNLLKKIIRRAIEISDVKVYAILNKLGLKEKDKIKSNNGQDEDNSVITTIIKDDILSAVKDNQSHLKADKNHSTKQKDTIKTTLLKKLMCSMQHPPSWLIHWFNLYTKLNNILTQYRSNEVKNHGFILIDNQTLSGFQFILNQYGCIVYHKELKRITVTTYNQFLTWKDISLSRLNVCLITWISNCLNTLNKSLGLRCGFNNVILTQLFLYGDCILKLFHNEGFYIIKEVEGFIMSLILNITEEDQFRKRFYNSMLNNITDAANKAQKNLLSRVCHTLLDKTVSDNIINGRWIILLSKFLKLIKLAGDNNLNNLSELYFLFRIFGHPMVDERQAMDAVKVNCNETKFYLLSSLSMLRGAFIYRIIKGFVNNYNRWPTLRNAIVLPLRWLTYYKLNTYPSLLELTERDLIVLSGLRFYREFRLPKKVDLEMIINDKAISPPKNLIWTSFPRNYMPSHIQNYIEHEKLKFSESDKSRRVLEYYLRDNKFNECDLYNCVVNQSYLNNPNHVVSLTGKERELSVGRMFAMQPGMFRQVQILAEKMIAENILQFFPESLTRYGDLELQKILELKAGISNKSNRYNDNYNNYISKCSIITDLSKFNQAFRYETSCICSDVLDELHGVQSLFSWLHLTIPHVTIICTYRHAPPYIRDHIVDLNNVDEQSGLYRYHMGGIEGWCQKLWTIEAISLLDLISLKGKFSITALINGDNQSIDISKPVRLMEGQTHAQADYLLALNSLKLLYKEYAGIGHKLKGTETYISRDMQFMSKTIQHNGVYYPASIKKVLRVGPWINTILDDFKVSLESIGSLTQELEYRGESLLCSLIFRNVWLYNQIALQLKNHALCNNKLYLDILKVLKHLKTFFNLDNIDTALTLYMNLPMLFGGGDPNLLYRSFYRRTPDFLTEAIVHSVFILSYYTNHDLKDKLQDLSDDRLNKFLTCIITFDKNPNAEFVTLMRDPQALGSERQAKITSEINRLAVTEVLSTAPNKIFSKSAQHYTTTEIDLNDIMQNIEPTYPHGLRVVYESLPFYKAEKIVNLISGTKSITNILEKTSAIDLTDIDRATEMMRKNITLLIRILPLDCNRDKREILSMENLSITELSKYVRERSWSLSNIVGVTSPSIMYTMDIKYTTSTIASGIIIEKYNVNSLTRGERGPTKPWVGSSTQEKKTMPVYNRQVLTKKQRDQIDLLAKLDWVYASIDNKDEFMEELSIGTLGLTYEKAKKLFPQYLSVNYLHRLTVSSRPCEFPASIPAYRTTNYHFDTSPINRILTEKYGDEDIDIVFQNCISFGLSLMSVVEQFTNVCPNRIILIPKLNEIHLMKPPIFTGDVDIHKLKQVIQKQHMFLPDKISLTQYVELFLSNKTLKSGSHVNSNLILAHKISDYFHNTYILSTNLAGHWILIIQLMKDSKGIFEKDWGEGYITDHMFINLKVFFNAYKTYLLCFHKGYGKAKLECDMNTSDLLCVLELIDSSYWKSMSKVFLEQKVIKYILSQDASLHRVKGCHSFKLWFLKRLNVAEFTVCPWVVNIDYHPTHMKAILTYIDLVRMGLINIDRIHIKNKHKFNDEFYTSNLFYINYNFSDNTHLLTKHIRIANSELENNYNKLYHPTPETLENILANPIKSNDKKTLNDYCIGKNVDSIMLPLLSNKKLVKSSAMIRTNYSKQDLYNLFPTVVIDRIIDHSGNTAKSNQLYTTTSHQISLVHNSTSLYCMLPWHHINRFNFVFSSTGCKISIEYILKDLKIKDPNCIAFIGEGAGNLLLRTVVELHPDIRYIYRSLKDCNDHSLPIEFLRLYNGHINIDYGENLTIPATDATNNIHWSYLHIKFAEPISLFVCDAELPVTVNWSKIIIEWSKHVRKCKYCSSVNKCTLIVKYHAQDDIDFKLDNITILKTYVCLGSKLKGSEVYLVLTIGPANIFPVFNVVQNAKLILSRTKNFIMPKKADKESIDANIKSLIPFLCYPITKKGINTALSKLKSVVSGDILSYSIAGRNEVFSNKLINHKHMNILKWFNHVLNFRSTELNYNHLYMVESTYPYLSELLNSLTTNELKKLIKITGSLLYNFHNE

SEQ ID NO: 7 - protein, 194 aa, respiratory syncytial virus
MSRRNPCKFEIRGHCLNGKRCHFSHNYFEWPPHALLVRQNFMLNRILKSMDKSIDTLSEISGAAELDRTEEYALGVVGVLESYIGSINNITKQSACVAMSKLLTELNSDDIKKLRDNEELNSPKIRVYNTVISYIESNRKNNKQTIHLLKRLPADVLKKTIKNTLDIHKSITINNPKELTVSDTNDHAKNNDTT

SEQ ID NO: 8 - protein, 90 aa, respiratory syncytial virus
MTMPKIMILPDKYPCSITSILITSRCRVTMYNRKNTLYFNQNNPNNHMYSPNQTFNEIHWTSQDLIDTIQNFLQHLGVIEDIYTIYILVS

SEQ ID NO: 9 - protein, 241 aa, respiratory syncytial virus
MEKFAPEFHGEDANNRATKFLESIKGKFTSPKDPKKKDSIISVNSIDIEVTKESPITSNSTIINPTNETDDNAGNKPNYQRKPLVSFKEDPIPSDNPFSKLYKETIETFDNNEEESSYSYEEINDQTNDNITARLDRIDEKLSEILGMLHTLVVASAGPTSARDGIRDAMVGLREEMIEKIRTEALMTNDRLEAMARLRNEESEKMAKDTSDEVSLNPTSEKLNNLLEGNDSDNDLSLEDF

SEQ ID NO: 10 - protein, 139 aa, respiratory syncytial virus
MGSNSLSMIKVRLQNLFDNDEVALLKITCYTDKLIHLTNALAKAVIHTIKLNGIVFVHVITSSDICPNNNIVVKSNFTTMPVLQNGGYIWEMMELTHCSQPNGLIDDNCEIKFSKKLSDSTMTNYMNQLSELLGFDLNP

SEQ ID NO: 11 - protein, 124 aa, respiratory syncytial virus
MDTTHNDTTPQRLMITDMRPLSLETTITSLTRDIITHRFIYLINHECIVRKLDERQATFTFLVNYEMKLLHKVGSTKYKKYTEYNTKYGTFPMPIFINHDGFLECIGIKPTKHTPIIYKYDLNP

SEQ ID NO: 12 - RNA, 1725 nt, respiratory syncytial virus
  source 1..1725: mol_type = unassigned RNA
atggagttgccaatcctcaaagcaaatgcaattaccacaatcctcgctgcagtcacattttgctttgcttctagtcaaaacatcactgaagaattttatcaatcaacatgcagtgcagttagcaaaggctatcttagtgctctaagaactggttggtatactagtgttataactatagaattaagtaatatcaaggaaaataagtgtaatggaacagatgctaaggtaaaattgataaaccaagaattagataaatataaaaatgctgtaacagaattgcagttgctcatgcaaagcacaacagcagcaaacaatcgagccagaagagaactaccaaggtttatgaattatacactcaacaataccaaaaaaaccaatgtaacattaagcaagaaaaggaaaagaagatttcttggttttttgttaggtgttggatctgcaatcgccagtggcattgctgtatctaaggtcctgcacttagaaggagaagtgaacaagatcaaaagtgctctactatccacaaacaaggccgtagtcagcttatcaaatggagttagtgtcttaaccagcaaagtgttagacctcaaaaactatatagataaacaattgttacctattgtgaataagcaaagctgcagaatatcaaatatagaaactgtgatagagttccaacaaaagaacaacagactactagagattaccagggaatttagtgttaatgcaggtgtaactacacctgtaagcacttacatgttaactaatagtgaattattgtcattaatcaatgatatgcctataacaaatgatcagaaaaagttaatgtccaacaatgttcaaatagttagacagcaaagttactctatcatgtccataataaaagaggaagtcttagcatatgtagtacaattaccactatatggtgtgatagatacaccttgttggaaattacacacatcccctctatgtacaaccaacacaaaagaagggtcaaacatctgtttaacaagaactgacagaggatggtactgtgacaatgcaggatcagtatctttcttcccacaagctgaaacatgtaaagttcaatcgaatcgagtattttgtgacacaatgaacagtttaacattaccaagtgaagtaaatctctgcaatgttgacatattcaatcccaaatatgattgtaaaattatgacttcaaaaacagatgtaagcagctccgttatcacatctctaggagccattgtgtcatgctatggcaaaactaaatgtacagcatccaataaaaatcgtggaatcataaagacattttctaacgggtgtgattatgtatcaaataaaggggtggacactgtgtctgtaggtaacacattatattatgtaaataagcaagaaggcaaaagtctctatgtaaaaggtgaaccaataataaatttctatgacccattagtattcccctctgatgaatttgatgcatcaatatctcaagtcaatgagaagattaaccagagtttagcatttattcgtaaatccgatgaattattacatcatgtaaatgctggtaaatcaaccacaaatatcatgataactactataattatagtgattatagtaatattgttatcattaattgctgttggactgctcctatactgtaaggccagaagcacaccagtcacactaagcaaggatcaactgagtggtataaataatattgcatttagtaactga

SEQ ID NO: 13 - RNA, 897 nt, respiratory syncytial virus
  source 1..897: mol_type = unassigned RNA
atgtccaaaaacaaggaccaacgcaccgctaagacactagaaaagacctgggacactctcaatcatttattattcatatcatcgggcttatataagttaaatcttaaatctatagcacaaatcacattatccattctggcaatgataatctcaacttcacttataattacagccatcatattcatagcctcggcaaaccacaaagtcacactaacaactgcaatcatacaagatgcaacaagccagatcaagaacacaaccccaacatacctcactcaggatcctcagcttggaatcagcttctccaatctgtctgaaattacatcacaaaccaccaccatactagcttcaacaacaccaggagtcaagtcaaacctgcaacccacaacagtcaagactaaaaacacaacaacaacccaaacacaacccagcaagcccactacaaaacaacgccaaaacaaaccaccaaacaaacccaataatgattttcacttcgaagtgtttaactttgtaccctgcagcatatgcagcaacaatccaacctgctgggctatctgcaaaagaataccaaacaaaaaaccaggaaagaaaaccaccaccaagcctacaaaaaaaccaaccttcaagacaaccaaaaaagatctcaaacctcaaaccactaaaccaaaggaagtacccaccaccaagcccacagaagagccaaccatcaacaccaccaaaacaaacatcacaactacactgctcaccaacaacaccacaggaaatccaaaactcacaagtcaaatggaaaccttccactcaacctcctccgaaggcaatctaagcccttctcaagtctccacaacatccgagcacccatcacaaccctcatctccacccaacacaacacgccagtag

SEQ ID NO: 14 - RNA, 195 nt, respiratory syncytial virus
  source 1..195: mol_type = unassigned RNA
atggaaaatacatccataacaatagaattctcaagcaaattctggccttactttacactaatacacatgatcacaacaataatctctttgctaatcataatctccatcatgactgcaatactaaacaaactttgtgaatataacgtattccataacaaaacctttgagttaccaagagctcgagtcaacacatag

SEQ ID NO: 15 - RNA, 771 nt, respiratory syncytial virus
  source 1..771: mol_type = unassigned RNA
atggaaacatacgtgaacaagcttcacgaaggctccacatacacagctgctgttcaatacaatgtcctagaaaaagacgatgaccctgcatcacttacaatatgggtgcccatgttccaatcatctatgccagcagatttacttataaaagaactagctaatgtcaacatactagtgaaacaaatatccacacccaagggaccttcactaagagtcatgataaactcaagaagtgcattgctagcacaaatgcccagcaaatttaccatatgtgctaatgtgtccttggatgaaagaagcaaactggcatatgatgtaaccacaccctgtgaaatcaaggcatgtagtctaacatgcctaaaatcaaaaaatatgttaactacagttaaagatctcactatgaagacactcaaccccacacatgatattattgctttatgtgaatttgaaaacatagtaacatcaaaaaaagtcataataccaacatacctaagatccatcagtgtcagaaataaagatctgaacacacttgaaaatataacaaccactgaattcaaaaatgccatcacaaatgcaaaaatcatcccttactcaggattactattagtcatcacagtgactgacaacaaaggagcattcaaatacataaagccgcaaagtcaattcatagtagatcttggagcttacctagaaaaagaaagtatatattatgttaccacaaattggaagcacacagctacacgatttgcaatcaaacccatggaagattaa

SEQ ID NO: 16 - RNA, 1176 nt, respiratory syncytial virus
  source 1..1176: mol_type = unassigned RNA
atggctcttagcaaagtcaagttgaatgatacactcaacaaagatcaacttctgtcatctagcaaatacaccatccaacggagcacaggagatagtattgatactcctaattatgatgtgcagaaacacatcaataagttatgtggcatgttattaatcacagaagatgctaatcataaattcactgggttaataggtatgttatatgctatgtctaggttaggaagagaagacaccataaaaatactcagagatgcgggatatcatgtaaaagcaaatggagtagatgtaacaacacatcgtcaagacatcaatgggaaagaaatgaaatttgaagtgttaacattggcaagcttaacaactgaaattcaaatcaacattgagatagaatctagaaaatcctacaaaaaaatgctaaaagaaatgggagaggtagctccagaatacaggcatgattctcctgattgtgggatgataatattatgtatagcagcattagtaataaccaaattggcagcaggggatagatctggtcttacagccgtgattaggagagctaataatgtcctaaaaaatgaaatgaaacgttacaaaggcttactacccaaggatatagccaacagcttctatgaagtgtttgaaaaacatccccactttatagatgtttttgttcattttggtatagcacaatcttccaccagaggtggcagtagagttgaagggatttttgcaggattgtttatgaatgcctatggtgcagggcaagtaatgctacggtggggagtcttagcaaaatcagttaaaaatattatgttaggacatgctagtgtgcaagcagaaatggaacaagttgttgaggtttatgaatatgcccaaaaattgggtggagaagcaggattctaccatatattgaacaacccaaaagcatcattattatctttgactcaatttcctcacttttccagtgtagtattaggcaatgctgctggcctaggcataatgggagagtacagaggtacaccgaggaatcaagatctatatgatgcagcaaaggcatatgctgaacaactcaaagaaaatggtgtgattaactacagtgtattagacttgacagcagaagaactagaggctatcaaacatcagcttaatccaaaagataatgatgtagagctttga

SEQ ID NO: 17 - RNA, 6498 nt, respiratory syncytial virus
  source 1..6498: mol_type = unassigned RNA
atggatcccattattaatggaaattctgctaatgtttatctaaccgatagttatttaaaaggtgttatctctttctcagagtgtaatgctttaggaagttacatattcaatggtccttatctcaaaaatgattataccaacttaattagtagacaaaatccattaatagaacacatgaatctaaagaaactaaatataacacagtccttaatatctaagtatcataaaggtgaaataaaattagaagagcctacttattttcagtcattacttatgacatacaagagtatgacctcgttggaacagattgctaccactaatttacttaaaaagataataagaagagctatagaaataagtgatgtcaaagtctatgctatattgaataaactagggcttaaagaaaaggacaagattaaatccaacaatggacaggatgaagacaactcagttattacgaccataatcaaagatgatatactttcagctgttaaggataatcaatctcatcttaaagcagacaaaaatcactctacaaaacaaaaagacacaatcaaaacaacactcttgaagaaattaatgtgttcaatgcagcatcctccatcatggttaatacattggtttaatttatacacaaaattaaacaacatattaacacagtatcgatcaaatgaggttaaaaaccatgggtttatattgatagataatcaaactcttagtggatttcaatttattttgaatcaatatggttgtatagtttatcataaggaactcaaaagaattactgtgacaacctataatcaattcttgacatggaaagatattagccttagtagattaaatgtttgtttaattacatggattagtaactgcttgaacacattaaataaaagcttaggcttaagatgcggattcaataatgttatcttgacacaactattcctttatggtgattgtatactaaagctatttcacaatgaggggttctacataataaaagaggtagagggatttattatgtctctaattttaaatataacagaagaagatcaattcagaaaacgattttataatagtatgctcaacaacatcacagatgctgctaataaagctcagaaaaatctgctatcaagagtatgtcatacattattagataagacagtatccgataatataataaatggcagatggataattctattaagtaagttccttaaattaattaagcttgcaggtgacaataaccttaacaatctgagtgaactatattttttgttcagaatatttggacacccaatggtagatgaaagacaagccatggatgctgttaaagttaattgcaatgagaccaaattttacttgttaagcagtttgagtatgttaagaggtgcctttatatatagaattataaaagggtttgtaaataattacaacagatggcctactttaagaaatgctattgttttacccttaagatggttaacttactataaactaaacacttatccttctttgttggaacttacagaaagagatttgattgtgttatcaggactacgtttctatcgtgagtttcggttgcctaaaaaagtggatcttgaaatgattataaatgataaagctatatcaccccctaaaaatttgatatggactagtttccctagaaattatatgccgtcacacatacaaaactatatagaacatgaaaaattaaaattttccgagagtgataaatcaagaagagtattagagtattatttaagagataacaaattcaatgaatgtgatttatacaactgtgtagttaatcaaagttatctcaacaaccctaatcatgtggtatcattgacaggcaaagaaagagaactcagtgtaggtagaatgtttgcaatgcaaccgggaatgttcagacaggttcaaatattggcagagaaaatgatagctgaaaacattttacaattctttcctgaaagtcttacaagatatggtgatctagaactacaaaaaatattagaattgaaagcaggaataagtaacaaatcaaatcgctacaatgataattacaacaattacattagtaagtgctctatcatcacagatctcagcaaattcaatcaagcatttcgatatgaaacgtcatgtatttgtagtgatgtgctggatgaactgcatggtgtacaatctctattttcctggttacatttaactattcctcatgtcacaataatatgcacatataggcatgcacccccctatataagagatcatattgtagatcttaacaatgtagatgaacaaagtggattatatagatatcacatgggtggtattgaagggtggtgtcaaaaactatggaccatagaagctatatcactattggatctaatatctctcaaagggaaattctcaattactgctttaattaatggtgacaatcaatcaatagatataagcaaaccagtcagactcatggaaggtcaaactcatgctcaagcagattatttgctagcattaaatagccttaaattactgtataaagagtatgcaggcataggtcacaaattaaaaggaactgagacttatatatcacgagatatgcaatttatgagtaaaacaattcaacataacggtgtatattaccctgctagtataaagaaagtcctaagagtgggaccgtggataaacactatacttgatgatttcaaagtgagtctagaatctataggtagtttgacacaagaattagaatatagaggtgaaagtctattatgcagtttaatatttagaaatgtatggttatataatcaaattgctctacaattaaaaaatcatgcgttatgtaacaataaattatatttggacatattaaaggttctgaaacacttaaaaaccttttttaatcttgataatattgatacagcattaacattgtatatgaatttacccatgttatttggtggtggtgatcccaacttgttatatcgaagtttctatagaagaactcctgatttcctcacagaggctatagttcactctgtgttcatacttagttattatacaaaccatgacttaaaagataaacttcaagatttgtcagatgatagattgaataagttcttaacatgcataatcacgtttgacaaaaaccctaatgctgaattcgtaacattgatgagagatcctcaagctttagggtctgagagacaagctaaaattactagtgaaatcaatagactggcagttacagaggttttgagtacagctccaaacaaaatattctccaaaagtgcacaacattataccactacagagatagatctaaatgatattatgcaaaatatagaacctacatatcctcacgggctaagagttgtttatgaaagtttacccttttataaagcagagaaaatagtaaatcttatatcaggtacaaaatctataactaacatactggaaaagacttctgccatagacttaacagatattgatagagccactgagatgatgaggaaaaacataactttgcttataaggatacttccattggattgtaacagagataaaagagaaatattgagtatggaaaacctaagtattactgaattaagcaaatatgttagggaaagatcttggtctttatccaatatagttggtgttacatcacccagtatcatgtatacaatggacatcaaatatacaacaagcactatagctagtggcataattatagagaaatataatgttaacagtttaacacgtggtgagagaggaccaactaaaccatgggttggttcatctacacaagagaaaaaaacaatgccagtttataatagacaagttttaaccaaaaaacaaagagatcaaatagatctattagcaaaattggattgggtgtatgcatctatagataacaaggatgaattcatggaagaactcagcataggaacccttgggttaacatatgaaaaggccaaaaaattatttccacaatatttaagtgtcaactatttgcatcgccttacagtcagtagtagaccatgtgaattccctgcatcaataccagcttatagaacaacaaattatcactttgacactagccctattaatcgcatattaacagaaaagtatggtgatgaagatattgacatagtattccaaaactgtataagctttggccttagcttaatgtcagtagtagaacaatttactaatgtatgtcctaacagaattattctcatacctaagcttaatgagatacatttgatgaaacctcccatattcacaggtgatgttgatattcacaagttaaaacaagtgatacaaaaacagcatatgtttttaccagacaaaataagtttgactcaatatgtggaattattcttaagtaacaaaacactcaaatctggatctcatgttaattctaatttaatattggcacataaaatatctgactattttcataatacttacattttaagtactaatttagctggacattggattctaattatacaacttatgaaagattctaaaggtatttttgaaaaagattggggagagggatatataactgatcatatgtttattaatttgaaagttttcttcaatgcttataagacctatctcttgtgttttcataaaggttatggcaaagcaaaactggagtgtgatatgaacacttcagatcttctatgtgtattggaattaatagacagtagttattggaagtctatgtctaaggtatttttagaacaaaaagttatcaaatacattcttagccaagatgcaagtttacatagagtaaaaggatgtcatagcttcaaattatggtttcttaaacgtcttaatgtagcagaatttacagtttgcccttgggttgttaacatagattatcatccaacacatatgaaagcaatattaacttatatagatcttgttagaatgggattgataaatatagatagaatacacattaaaaataaacacaaattcaatgatgaattttatacttctaatctcttttacattaattataacttctcagataatactcatctattaactaaacatataaggattgctaattcagaattagaaaataattacaacaaattatatcatcctacaccagaaaccctagagaatatactagccaatccgattaaaagtaatgacaaaaagacactgaacgactattgtataggtaaaaatgttgactcaataatgttaccattgttatctaataagaagcttgttaaatcgtctgcaatgattagaaccaattacagcaaacaagacctgtacaatctattccctacggttgtgatcgatagaattatagatcattcaggtaatacagccaaatccaaccaactttacactactacttcccatcaaatatctttagtgcacaatagcacatcactttattgcatgcttccttggcatcatattaatagattcaattttgtatttagttctacaggttgtaaaattagtatagagtatattttaaaagaccttaaaattaaagatcctaattgtatagcattcataggtgaaggagcagggaatttattattgcgtacagtggtggaacttcatcctgacataagatatatttacagaagtctgaaagattgcaatgatcatagtttacctattgagtttttaaggctatacaatggacatatcaacattgattatggtgaaaatttgaccattcctgctacagatgcaaccaacaacattcattggtcttatttacatataaagtttgctgaacctatcagtctttttgtatgtgatgccgaattgcctgtaacagtcaactggagtaaaattataatagaatggagcaagcatgtaagaaaatgcaagtactgttcctcagttaataaatgtacgttaatagtaaaatatcatgctcaagatgatattgatttcaaattagacaatataactatattaaaaacttatgtatgcttaggcagtaagttaaagggatcggaggtttacttagtccttacaataggtcctgcaaatatatttccagtatttaatgtagtacaaaatgctaaattgatactatcaagaaccaaaaatttcatcatgcctaagaaagctgataaagagtctattgatgcaaatattaaaagtttgataccctttctttgttaccctataacaaaaaaaggaattaatactgcattgtcaaaactaaagagtgttgttagtggagatatactatcatattctatagctggacggaatgaagttttcagcaataaacttataaatcataagcatatgaacatcttaaagtggttcaatcatgttttaaatttcagatcaacagaactaaactataaccatttatatatggtagaatctacatatccttacctaagtgaattgttaaacagcttgacaactaatgaacttaaaaaactgattaaaatcacaggtagtctgttatacaactttcataatgaataa

SEQ ID NO: 18 - RNA, 585 nt, respiratory syncytial virus
  source 1..585: mol_type = unassigned RNA
atgtcacgaaggaatccttgcaaatttgaaattcgaggtcattgcttgaatggtaagagatgtcattttagtcataattattttgaatggccaccccatgcactgctcgtaagacaaaactttatgttaaacagaatacttaagtctatggataaaagtatagataccttatcagaaataagtggagctgcagagttggacagaacagaagagtatgctcttggtgtagttggagtgctagagagttatataggatcaataaataatataactaaacaatcagcatgtgttgccatgagcaaactcctcactgaactcaatagtgatgatatcaaaaaactgagagacaatgaagagctaaattcacccaagataagagtgtacaatactgtcatatcatatattgaaagcaacaggaaaaacaataaacaaactatccatctgttaaaaagattgccagcagacgtattgaagaaaaccatcaaaaacacattggatatccacaagagcataaccatcaacaacccaaaagaattaactgttagtgatacaaatgaccatgccaaaaataatgatactacctga

SEQ ID NO: 19 - RNA, 273 nt, respiratory syncytial virus
  source 1..273: mol_type = unassigned RNA
atgaccatgccaaaaataatgatactacctgacaaatatccttgtagtataacttccatactaataacaagtagatgtagagtcactatgtataatcgaaagaacacactatatttcaatcaaaacaacccaaataaccatatgtactcaccgaatcaaacattcaatgaaatccattggacctcacaagacttgattgacacaattcaaaattttctacagcatctaggtgttattgaggatatatatacaatatatatattagtgtcataa

SEQ ID NO: 20 - RNA, 726 nt, respiratory syncytial virus
  source 1..726: mol_type = unassigned RNA
atggaaaagtttgctcctgaattccatggagaagatgcaaacaacagggctactaaattcctagaatcaataaagggcaaattcacatcacctaaagatcccaagaaaaaagatagtatcatatctgtcaactcaatagatatagaagtaaccaaagaaagccctataacatcaaattcaaccattattaacccaacaaatgagacagatgataatgcagggaacaagcccaattatcaaagaaaacctctagtaagtttcaaagaagaccctataccaagtgataatcccttttcaaaactatacaaagaaaccatagagacatttgataacaatgaagaagaatctagctattcatatgaagaaataaatgatcagacgaacgataatataactgcaagattagataggattgatgaaaaattaagtgaaatactaggaatgcttcacacattagtagtagcaagtgcaggacctacatctgctagggatggtataagagatgccatggttggtttaagagaagaaatgatagaaaaaatcagaactgaagcattaatgaccaatgacagattagaagctatggcaagactcaggaatgaggaaagtgaaaagatggcaaaagacacatcagatgaagtgtctctcaatccaacatcagagaaattgaacaacctgttggaagggaatgatagtgacaatgatctatcacttgaagatttctga

SEQ ID NO: 21 - RNA, 420 nt, respiratory syncytial virus
  source 1..420: mol_type = unassigned RNA
atgggcagcaattcgttgagtatgataaaagttagattacaaaatttgtttgacaatgatgaagtagcattgttaaaaataacatgctatactgacaaattaatacatttaactaatgctttggctaaggcagtgatacatacaatcaaattgaatggcattgtgtttgtgcatgttattacaagtagtgatatttgccctaataataatattgtagtaaaatccaatttcacaacaatgccagtgctacaaaatggaggttatatatgggaaatgatggaattaacacattgctctcaacctaatggtctaatagatgacaattgtgaaattaaattctccaaaaaactaagtgattcaacaatgaccaattatatgaatcaattatctgaattacttggatttgatcttaatccataa

SEQ ID NO: 22 - RNA, 375 nt, respiratory syncytial virus
  source 1..375: mol_type = unassigned RNA
atggacacaacccacaatgataccacaccacaaagactgatgatcacagacatgagaccgttgtcacttgagactacaataacatcactaaccagagacatcataacacacagatttatatacttaataaatcatgaatgcatagtgagaaaacttgatgaaagacaggccacatttacattcctggtcaactatgaaatgaaactattgcacaaagtaggaagcactaaatataaaaaatatactgaatacaacacaaaatatggcactttccctatgccgatattcatcaatcatgatgggttcttagaatgcattggcattaagcctacaaagcatactcccataatatacaagtatgatctcaatccatag

SEQ ID NO: 23 - DNA, 42 bp, Homo sapiens
  source 1..42: mol_type = unassigned DNA
ggcgctgcctacggaggtggcagccatctccttctcggcatc

SEQ ID NO: 24 - DNA, 186 bp, Homo sapiens
  source 1..186: mol_type = unassigned DNA
catcacatttaaaagcatctcagcctaccatgagaataagagaaagaaaatgaagatcaaaagcttattcatctgtttttctttttcgttggtgtaaagccaacaccctgtctaaaaaacataaatttctttaatcattttgcctcttttctctgtgcttcaattaataaaaaatggaaagaatct

SEQ ID NO: 25 - DNA, 186 bp, Homo sapiens
  source 1..186: mol_type = unassigned DNA
catcacatttaaaagcatctcagcctaccatgagaataagagaaagaaaatgaagatcaatagcttattcatctctttttctttttcgttggtgtaaagccaacaccctgtctaaaaaacataaatttctttaatcattttgcctcttttctctgtgcttcaattaataaaaaatggaaagaacct

SEQ ID NO: 26 - DNA, 110 bp, Homo sapiens
  source 1..110: mol_type = unassigned DNA
gctggagcctcggtggccatgcttcttgccccttgggcctccccccagcccctcctccccttcctgcacccgtacccccgtggtctttgaataaagtctgagtgggcggc

SEQ ID NO: 27 - DNA, 108 bp, Homo sapiens
  source 1..108: mol_type = unassigned DNA
gctggagcctcggtagccgttcctcctgcccgctgggcctcccaacgggccctcctcccctccttgcaccggcccttcctggtctttgaataaagtctgagtgggcag

SEQ ID NO: 28 - DNA, 132 bp, Homo sapiens
  source 1..132: mol_type = unassigned DNA
gctcgctttcttgctgtccaatttctattaaaggttcctttgttccctaagtccaactactaaactgggggatattatgaagggccttgagcatctggattctgcctaataaaaaacatttattttcattgc

SEQ ID NO: 29 - DNA, 44 bp, synthetic construct
  misc_feature 1..44: note = Center, alpha-complex-binding portion of the 3'UTR of an alpha-globin gene (muag)
  source 1..44: mol_type = other DNA
gcccgatgggcctcccaacgggccctcctcccctccttgcaccg

SEQ ID NO: 30 - DNA, 24 bp, synthetic construct
  misc_feature 1..24: note = particular preferred histone stem-loop sequence
  source 1..24: mol_type = other DNA
caaaggctcttttcagagccacca

SEQ ID NO: 31 - RNA, 1942 nt, synthetic construct
  misc_feature 1..1942: note = RSV-F long (GC) R1691
  source 1..1942: mol_type = other RNA
gggagaaagcttaccatggagctgcccatcctcaaggccaacgccatcaccaccatcctggcggccgtgacgttctgcttcgccagctcccagaacatcaccgaggagttctaccagagcacctgctccgccgtcagcaagggctacctgtccgccctccggaccgggtggtacacgagcgtgatcaccatcgagctgtccaacatcaaggagaacaagtgcaacggcaccgacgcgaaggtgaagctgatcaaccaggagctcgacaagtacaagaacgccgtcaccgagctgcagctgctcatgcagagcacgaccgccgccaacaaccgcgcgcggcgcgagctgccgcggttcatgaactacaccctgaacaacaccaagaagacgaacgtgaccctctccaagaagcgcaagcggcgcttcctggggttcctgctcggcgtggggagcgccatcgcctccggcatcgccgtcagcaaggtgctgcacctggagggcgaggtgaacaagatcaagtccgccctcctgagcaccaacaaggcggtcgtgtccctgagcaacggggtgtccgtcctcaccagcaaggtgctggacctgaagaactacatcgacaagcagctcctgcccatcgtgaacaagcagtcctgccggatcagcaacatcgagacggtcatcgagttccagcagaagaacaaccgcctgctcgagatcacccgggagttcagcgtgaacgccggcgtgaccacccccgtctccacgtacatgctgaccaacagcgagctgctctccctgatcaacgacatgcccatcaccaacgaccagaagaagctgatgagcaacaacgtgcagatcgtgcgccagcagtcctacagcatcatgtccatcatcaaggaggaggtcctcgcctacgtggtgcagctgccgctgtacggggtcatcgacaccccctgctggaagctccacacgagccccctgtgcaccaccaacaccaaggagggctccaacatctgcctgacgcggaccgaccgcgggtggtactgcgacaacgccggcagcgtgtccttcttcccccaggccgagacctgcaaggtccagagcaaccgggtgttctgcgacaccatgaactccctcacgctgccgagcgaggtgaacctgtgcaacgtcgacatcttcaaccccaagtacgactgcaagatcatgacctccaagaccgacgtgagctccagcgtgatcacctccctcggcgcgatcgtcagctgctacgggaagacgaagtgcaccgccagcaacaagaaccgcggcatcatcaagaccttctccaacgggtgcgactacgtgagcaacaagggcgtggacaccgtctccgtgggcaacaccctgtactacgtgaacaagcaggaggggaagagcctgtacgtcaagggcgagcccatcatcaacttctacgaccccctcgtgttcccgtccgacgagttcgacgccagcatctcccaggtgaacgagaagatcaaccagagcctggccttcatccggaagtccgacgagctgctgcaccacgtcaacgccgggaagagcacgaccaacatcatgatcaccaccatcatcatcgtgatcatcgtgatcctcctgtccctgatcgcggtcggcctcctgctgtactgcaaggcccgcagcacgcccgtgaccctctccaaggaccagctgagcgggatcaacaacatcgccttctccaactgaggactagttataagactgactagcccgatgggcctcccaacgggccctcctcccctccttgcaccgagattaataaaaaaaaaaaaaaaaaaaaaaaaaaaaaaaaaaaaaaaaaaaaaaaaaaaaaaaaaaaaaaaatgcatcccccccccccccccccccccccccccccccaaaggctcttttcagagccaccagaatt

SEQ ID NO: 32 - RNA, 2107 nt, synthetic construct
  misc_feature 1..2107: note = RSV-F long (GC) R2510
  source 1..2107: mol_type = other RNA
ggggcgctgcctacggaggtggcagccatctccttctcggcatcaagcttaccatggagctgcccatcctcaaggccaacgccatcaccaccatcctggcggccgtgacgttctgcttcgccagctcccagaacatcaccgaggagttctaccagagcacctgctccgccgtcagcaagggctacctgtccgccctccggaccgggtggtacacgagcgtgatcaccatcgagctgtccaacatcaaggagaacaagtgcaacggcaccgacgcgaaggtgaagctgatcaaccaggagctcgacaagtacaagaacgccgtcaccgagctgcagctgctcatgcagagcacgaccgccgccaacaaccgcgcgcggcgcgagctgccgcggttcatgaactacaccctgaacaacaccaagaagacgaacgtgaccctctccaagaagcgcaagcggcgcttcctggggttcctgctcggcgtggggagcgccatcgcctccggcatcgccgtcagcaaggtgctgcacctggagggcgaggtgaacaagatcaagtccgccctcctgagcaccaacaaggcggtcgtgtccctgagcaacggggtgtccgtcctcaccagcaaggtgctggacctgaagaactacatcgacaagcagctcctgcccatcgtgaacaagcagtcctgccggatcagcaacatcgagacggtcatcgagttccagcagaagaacaaccgcctgctcgagatcacccgggagttcagcgtgaacgccggcgtgaccacccccgtctccacgtacatgctgaccaacagcgagctgctctccctgatcaacgacatgcccatcaccaacgaccagaagaagctgatgagcaacaacgtgcagatcgtgcgccagcagtcctacagcatcatgtccatcatcaaggaggaggtcctcgcctacgtggtgcagctgccgctgtacggggtcatcgacaccccctgctggaagctccacacgagccccctgtgcaccaccaacaccaaggagggctccaacatctgcctgacgcggaccgaccgcgggtggtactgcgacaacgccggcagcgtgtccttcttcccccaggccgagacctgcaaggtccagagcaaccgggtgttctgcgacaccatgaactccctcacgctgccgagcgaggtgaacctgtgcaacgtcgacatcttcaaccccaagtacgactgcaagatcatgacctccaagaccgacgtgagctccagcgtgatcacctccctcggcgcgatcgtcagctgctacgggaagacgaagtgcaccgccagcaacaagaaccgcggcatcatcaagaccttctccaacgggtgcgactacgtgagcaacaagggcgtggacaccgtctccgtgggcaacaccctgtactacgtgaacaagcaggaggggaagagcctgtacgtcaagggcgagcccatcatcaacttctacgaccccctcgtgttcccgtccgacgagttcgacgccagcatctcccaggtgaacgagaagatcaaccagagcctggccttcatccggaagtccgacgagctgctgcaccacgtcaacgccgggaagagcacgaccaacatcatgatcaccaccatcatcatcgtgatcatcgtgatcctcctgtccctgatcgcggtcggcctcctgctgtactgcaaggcccgcagcacgcccgtgaccctctccaaggaccagctgagcgggatcaacaacatcgccttctccaactgaggactagtgcatcacatttaaaagcatctcagcctaccatgagaataagagaaagaaaatgaagatcaatagcttattcatctctttttctttttcgttggtgtaaagccaacaccctgtctaaaaaacataaatttctttaatcattttgcctcttttctctgtgcttcaattaataaaaaatggaaagaacctagatctaaaaaaaaaaaaaaaaaaaaaaaaaaaaaaaaaaaaaaaaaaaaaaaaaaaaaaaaaaaaaaaatgcatcccccccccccccccccccccccccccccccaaaggctcttttcagagccaccagaatt

SEQ ID NO: 33 - RNA, 2044 nt, synthetic construct
  misc_feature 1..2044: note = RSV-Fdel554-574 long (GC) R2821
  source 1..2044: mol_type = other RNA
ggggcgctgcctacggaggtggcagccatctccttctcggcatcaagcttaccatggagctgcccatcctcaaggccaacgccatcaccaccatcctggcggccgtgacgttctgcttcgccagctcccagaacatcaccgaggagttctaccagagcacctgctccgccgtcagcaagggctacctgtccgccctccggaccgggtggtacacgagcgtgatcaccatcgagctgtccaacatcaaggagaacaagtgcaacggcaccgacgcgaaggtgaagctgatcaaccaggagctcgacaagtacaagaacgccgtcaccgagctgcagctgctcatgcagagcacgaccgccgccaacaaccgcgcgcggcgcgagctgccgcggttcatgaactacaccctgaacaacaccaagaagacgaacgtgaccctctccaagaagcgcaagcggcgcttcctggggttcctgctcggcgtggggagcgccatcgcctccggcatcgccgtcagcaaggtgctgcacctggagggcgaggtgaacaagatcaagtccgccctcctgagcaccaacaaggcggtcgtgtccctgagcaacggggtgtccgtcctcaccagcaaggtgctggacctgaagaactacatcgacaagcagctcctgcccatcgtgaacaagcagtcctgccggatcagcaacatcgagacggtcatcgagttccagcagaagaacaaccgcctgctcgagatcacccgggagttcagcgtgaacgccggcgtgaccacccccgtctccacgtacatgctgaccaacagcgagctgctctccctgatcaacgacatgcccatcaccaacgaccagaagaagctgatgagcaacaacgtgcagatcgtgcgccagcagtcctacagcatcatgtccatcatcaaggaggaggtcctcgcctacgtggtgcagctgccgctgtacggggtcatcgacaccccctgctggaagctccacacgagccccctgtgcaccaccaacaccaaggagggctccaacatctgcctgacgcggaccgaccgcgggtggtactgcgacaacgccggcagcgtgtccttcttcccccaggccgagacctgcaaggtccagagcaaccgggtgttctgcgacaccatgaactccctcacgctgccgagcgaggtgaacctgtgcaacgtcgacatcttcaaccccaagtacgactgcaagatcatgacctccaagaccgacgtgagctccagcgtgatcacctccctcggcgcgatcgtcagctgctacgggaagacgaagtgcaccgccagcaacaagaaccgcggcatcatcaagaccttctccaacgggtgcgactacgtgagcaacaagggcgtggacaccgtctccgtgggcaacaccctgtactacgtgaacaagcaggaggggaagagcctgtacgtcaagggcgagcccatcatcaacttctacgaccccctcgtgttcccgtccgacgagttcgacgccagcatctcccaggtgaacgagaagatcaaccagagcctggccttcatccggaagtccgacgagctgctgcaccacgtcaacgccgggaagagcacgaccaacatcatgatcaccaccatcatcatcgtgatcatcgtgatcctcctgtccctgatcgcggtcggcctcctgctgtactgcaaggcccgctgaggactagtgcatcacatttaaaagcatctcagcctaccatgagaataagagaaagaaaatgaagatcaatagcttattcatctctttttctttttcgttggtgtaaagccaacaccctgtctaaaaaacataaatttctttaatcattttgcctcttttctctgtgcttcaattaataaaaaatggaaagaacctagatctaaaaaaaaaaaaaaaaaaaaaaaaaaaaaaaaaaaaaaaaaaaaaaaaaaaaaaaaaaaaaaaatgcatcccccccccccccccccccccccccccccccaaaggctcttttcagagccaccagaatt

SEQ ID NO: 34 - RNA, 1558 nt, synthetic construct
  misc_feature 1..1558: note = RSV-N (GC) R2831
  source 1..1558: mol_type = other RNA
ggggcgctgcctacggaggtggcagccatctccttctcggcatcaagcttaccatggccctgagcaaggtgaagctcaacgacaccctgaacaaggaccagctgctctccagctccaagtacaccatccagcgcagcacgggcgactccatcgacacccccaactacgacgtccagaagcacatcaacaagctgtgcgggatgctgctcatcaccgaggacgccaaccacaagttcaccggcctgatcgggatgctgtacgcgatgagccggctcggccgcgaggacacgatcaagatcctgcgggacgccgggtaccacgtgaaggccaacggcgtggacgtcaccacccaccgccaggacatcaacggcaaggagatgaagttcgaggtgctgaccctcgcctccctgacgaccgagatccagatcaacatcgagatcgagagccggaagtcctacaagaagatgctgaaggagatgggggaggtggccccggagtaccgccacgacagccccgactgcggcatgatcatcctctgcatcgcggccctggtcatcaccaagctggccgccggggaccggtccggcctcaccgcggtgatccgccgggccaacaacgtgctgaagaacgagatgaagcgctacaaggggctgctccccaaggacatcgccaacagcttctacgaggtcttcgagaagcacccccacttcatcgacgtgttcgtgcacttcggcatcgcccagtccagcacgcggggcgggtcccgcgtcgagggcatcttcgccgggctgttcatgaacgcgtacggcgccggccaggtgatgctgcggtggggcgtgctcgccaagagcgtcaagaacatcatgctggggcacgcctccgtgcaggccgagatggagcaggtggtcgaggtgtacgagtacgcgcagaagctgggcggcgaggccgggttctaccacatcctcaacaacccgaaggccagcctgctgtccctcacccagttcccgcacttcagcagcgtggtcctggggaacgccgccggcctggggatcatgggcgagtaccgcgggaccccgcggaaccaggacctctacgacgcggccaaggcctacgccgagcagctgaaggagaacggcgtgatcaactactccgtgctggacctcaccgccgaggagctggaggcgatcaagcaccagctgaaccccaaggacaacgacgtcgagctctgaggactagtgcatcacatttaaaagcatctcagcctaccatgagaataagagaaagaaaatgaagatcaatagcttattcatctctttttctttttcgttggtgtaaagccaacaccctgtctaaaaaacataaatttctttaatcattttgcctcttttctctgtgcttcaattaataaaaaatggaaagaacctagatctaaaaaaaaaaaaaaaaaaaaaaaaaaaaaaaaaaaaaaaaaaaaaaaaaaaaaaaaaaaaaaaatgcatcccccccccccccccccccccccccccccccaaaggctcttttcagagccaccagaatt

SEQ ID NO: 35 - RNA, 967 nt, synthetic construct
  misc_feature 1..967: note = RSV-M2-1 (GC) R2833
  source 1..967: mol_type = other RNA
ggggcgctgcctacggaggtggcagccatctccttctcggcatcaagcttaccatgagccgccggaacccctgcaagttcgagatccgcggccactgcctgaacgggaagcggtgccacttctcccacaactacttcgagtggccgccccacgccctcctggtgcgccagaacttcatgctgaaccggatcctcaagagcatggacaagtccatcgacaccctgagcgagatctccggcgccgcggagctggaccgcaccgaggagtacgccctcggggtcgtgggcgtgctggagagctacatcgggtccatcaacaacatcacgaagcagagcgcctgcgtcgccatgtccaagctgctcaccgagctgaacagcgacgacatcaagaagctgcgggacaacgaggagctcaactcccccaagatccgcgtgtacaacaccgtgatcagctacatcgagtccaaccggaagaacaacaagcagaccatccacctgctgaagcgcctccccgccgacgtcctgaagaagacgatcaagaacaccctggacatccacaagagcatcaccatcaacaacccgaaggagctcaccgtgtccgacacgaacgaccacgcgaagaacaacgacaccacctgaggactagtgcatcacatttaaaagcatctcagcctaccatgagaataagagaaagaaaatgaagatcaatagcttattcatctctttttctttttcgttggtgtaaagccaacaccctgtctaaaaaacataaatttctttaatcattttgcctcttttctctgtgcttcaattaataaaaaatggaaagaacctagatctaaaaaaaaaaaaaaaaaaaaaaaaaaaaaaaaaaaaaaaaaaaaaaaaaaaaaaaaaaaaaaaatgcatcccccccccccccccccccccccccccccccaaaggctcttttcagagccaccagaatt

SEQ ID NO: 36 - DNA, 75 bp, Homo sapiens
  source 1..75: mol_type = unassigned DNA
gcggctcggccattttgtcccagtcagtccggaggctgcggctgcagaagtaccgcctgcggagtaactgcaaag

SEQ ID NO: 37 - RNA, 24 nt, synthetic construct
  misc_feature 1..24: note = histone stem-loop sequence
  source 1..24: mol_type = other RNA
caaaggctcttttcagagccacca